European Patent Application EP 4 428 133 A1, published September 11, 2024. Title: Bifunctional protein targeting chimeras (PROTACs) comprising arylidene-indolinone scaffold as DCAF11 Ligand and use thereof. Applicant: Max-Planck-Gesellschaft zur Förderung der Wissenschaften e.V. The sequence listing filed with the application follows.

SEQUENCE LISTING (16 sequences)

SEQ ID NO: 1 - DNA, 22 bp, synthetic construct
  source 1..22: mol_type = other DNA; note = forward primer for PDE6D
gcagtccttgatagaggcagca

SEQ ID NO: 2 - DNA, 23 bp, synthetic construct
  source 1..23: mol_type = other DNA; note = reverse primer for PDE6D
gaaaagtctcactctggatgtgc

SEQ ID NO: 3 - DNA, 22 bp, synthetic construct
  source 1..22: mol_type = other DNA; note = forward primer for GAPDH
gtctcctctgacttcaacagcg

SEQ ID NO: 4 - DNA, 22 bp, synthetic construct
  source 1..22: mol_type = other DNA; note = reverse primer for GAPDH
accaccctgttgctgtagccaa

SEQ ID NO: 5 - DNA, 23 bp, synthetic construct
  source 1..23: mol_type = other DNA; note = forward primer for BRD2
cggcttatgttctccaactgcta

SEQ ID NO: 6 - DNA, 22 bp, synthetic construct
  source 1..22: mol_type = other DNA; note = reverse primer for BRD2
ggcagtagagactggtaaaggc

SEQ ID NO: 7 - DNA, 23 bp, synthetic construct
  source 1..23: mol_type = other DNA; note = forward primer for BRD3
ccaaccatcactgcaaacgtcac

SEQ ID NO: 8 - DNA, 22 bp, synthetic construct
  source 1..22: mol_type = other DNA; note = reverse primer for BRD3
ggagtggttgtgtctgctttcc

SEQ ID NO: 9 - DNA, 22 bp, synthetic construct
  source 1..22: mol_type = other DNA; note = forward primer for BRD4
cgctatgtcacctcctgtttgc

SEQ ID NO: 10 - DNA, 22 bp, synthetic construct
  source 1..22: mol_type = other DNA; note = reverse primer for BRD4
actctgaggacgagaagccctt

SEQ ID NO: 11 - DNA, 67 bp, synthetic construct
  source 1..67: mol_type = other DNA; note = forward primer BRD2 cDNA insertion into pOPIN-E vector
aggagatataccatggattacaaggatgacgacgataagggatctatgctgcaaaacgtgactcccc

SEQ ID NO: 12 - DNA, 44 bp, synthetic construct
  source 1..44: mol_type = other DNA; note = reverse primer for BRD2 cDNA insertion into pOPIN-E vector
gtgatggtgatgtttttagcctgagtctgaatcactggtgtctg

SEQ ID NO: 13 - DNA, 25 bp, synthetic construct
  source 1..25: mol_type = other DNA; note = forward primer for DCAF11 KO1
caccgagagttggagatcagatacc

SEQ ID NO: 14 - DNA, 25 bp, synthetic construct
  source 1..25: mol_type = other DNA; note = reverse primer for DCAF11 KO1
aaacggtatctgatctccaactctc

SEQ ID NO: 15 - DNA, 25 bp, synthetic construct
  source 1..25: mol_type = other DNA; note = forward primer for DCAF11 KO2
caccggatggacgagaagtactagg

SEQ ID NO: 16 - DNA, 25 bp, synthetic construct
  source 1..25: mol_type = other DNA; note = reverse primer for DCAF11 KO2
aaaccctagtacttctcgtccatcc